European Patent Application EP 4 721 767 A1, published April 8, 2026. Title: 抗B7-H3的抗体或其片段以及靶向B7-H3的抗体药物偶联物. Applicant: 江苏迈威康新药研发有限公司. The sequence listing filed with the application follows.

SEQUENCE LISTING (18 sequences)

SEQ ID NO: 1 - protein, 121 aa, synthetic construct
EVQLVQSGAEVKKPGASVKVSCKASGYTFTEYIMHWVRQAPGQGLEWMGGINPASGGTTYNQKFKGRVTMTRDTSISTAYMELSRLRSEDTAVYYCARKGKDYFDWYFDVWGQGTTVTVSS

SEQ ID NO: 2 - protein, 106 aa, synthetic construct
DIQLTQSPSSLSASVGDRVTMTCSASSSVSYMHWYQQKPGKAPKLLIYDTSKLASGVPSRFSGSGSGTDFTLTISSLQPEDFATYYCQQWSSNPLTFGGGTKVEIK

SEQ ID NO: 3 - protein, 106 aa, synthetic construct
DIQLTQSPSSLSASVGDRVTMTCSASSSVSYMHWYQQKPGKAPKLLIYDTSKLASGVPSRFSGSGSGTDFTLTISSLQPEDFATYYCQQWSSAPLTFGGGTKVEIK

SEQ ID NO: 4 - protein, 106 aa, synthetic construct
DIQLTQSPSSLSASVGDRVTMTCSASSSVSYMHWYQQKPGKAPKLLIYDTSKLASGVPSRFSGSGSGTDFTLTISSLQPEDFATYYCQQWSASPLTFGGGTKVEIK

SEQ ID NO: 5 - protein, 106 aa, synthetic construct
DIQLTQSPSSLSASVGDRVTMTCSASSSVSYMHWYQQKPGKAPKLLIYDTSKLASGVPSRFSGSGSGTDFTLTISSLQPEDFATYYCQQWSSQPLTFGGGTKVEIK

SEQ ID NO: 6 - protein, 106 aa, synthetic construct
DIQLTQSPSSLSASVGDRVTMTCSASSSVSYMHWYQQKPGKAPKLLIYDTSKLASGVPSRFSGSGSGTDFTLTISSLQPEDFATYYCQQWSSGPLTFGGGTKVEIK

SEQ ID NO: 7 - protein, 106 aa, synthetic construct
DIQLTQSPSSLSASVGDRVTMTCSASSSVSYMHWYQQKPGKAPKLLIYDTSKLASGVPSRFSGSGSGTDFTLTISSLQPEDFATYYCQQWSGSPLTFGGGTKVEIK

SEQ ID NO: 8 - protein, 5 aa, synthetic construct
EYIMH

SEQ ID NO: 9 - protein, 17 aa, synthetic construct
GINPASGGTTYNQKFKG

SEQ ID NO: 10 - protein, 12 aa, synthetic construct
KGKDYFDWYFDV

SEQ ID NO: 11 - protein, 10 aa, synthetic construct
SASSSVSYMH

SEQ ID NO: 12 - protein, 7 aa, synthetic construct
DTSKLAS

SEQ ID NO: 13 - protein, 9 aa, synthetic construct
QQWSSNPLT

SEQ ID NO: 14 - protein, 9 aa, synthetic construct
QQWSSAPLT

SEQ ID NO: 15 - protein, 9 aa, synthetic construct
QQWSASPLT

SEQ ID NO: 16 - protein, 9 aa, synthetic construct
QQWSSQPLT

SEQ ID NO: 17 - protein, 9 aa, synthetic construct
QQWSSGPLT

SEQ ID NO: 18 - protein, 9 aa, synthetic construct
QQWSGSPLT